European Patent Application EP 4 752 154 A1, published June 3, 2026. Title: 탄산탈수소효소 IX를 표적으로 하는 펩타이드 구조체 및 이들의 용도. Applicant: (주)씨바이오멕스. The sequence listing filed with the application follows.

SEQUENCE LISTING (107 sequences)

SEQ ID NO: 1 - protein, 5 aa, synthetic construct
  REGION 1..5: note = Synthetic Polypeptide
YRFRR

SEQ ID NO: 2 - protein, 4 aa, synthetic construct
  REGION 1..4: note = Synthetic Polypeptide
RFRR

SEQ ID NO: 3 - protein, 4 aa, synthetic construct
  REGION 1..4: note = Synthetic Polypeptide
RARR

SEQ ID NO: 4 - protein, 5 aa, synthetic construct
  REGION 1..5: note = Synthetic Polypeptide
YRARR

SEQ ID NO: 5 - protein, 5 aa, synthetic construct
  REGION 1..5: note = Synthetic Polypeptide
ARFRR

SEQ ID NO: 6 - protein, 5 aa, synthetic construct
  REGION 1..5: note = Synthetic Polypeptide
ARARR

SEQ ID NO: 7-8 - skipped (2 entries)

SEQ ID NO: 9 - protein, 4 aa, synthetic construct
  REGION 1..4: note = synthetic Polypeptide
RNRR

SEQ ID NO: 10 - protein, 4 aa, synthetic construct
  REGION 1..4: note = Synthetic Polypeptide
AAAA

SEQ ID NO: 11 - protein, 4 aa, synthetic construct
  REGION 1..4: note = Synthetic Polypeptide
RERR

SEQ ID NO: 12 - protein, 5 aa, synthetic construct
  REGION 1..5: note = Synthetic Polypeptide
  SITE 3: note = 2-amino-3-((2S,3R,4S,5R,6S)-3,4,5,6-tetrahydroxytetrahydro-2H-pyran-2-carboxamido)propanoic acid
YRXRR

SEQ ID NO: 13-14 - skipped (2 entries)

SEQ ID NO: 15 - protein, 5 aa, synthetic construct
  REGION 1..5: note = Synthetic Polypeptide
  SITE 3: note = 2-amino-3-((2S,3R,4S,5R,6S)-3,4,5,6-tetrahydroxytetrahydro-2H-pyran-2-carboxamido)propanoic acid
YSXRR

SEQ ID NO: 16 - protein, 5 aa, synthetic construct
  REGION 1..5: note = Synthetic Polypeptide
  SITE 3: note = 2-amino-3-((2S,3R,4S,5R,6S)-3,4,5,6-tetrahydroxytetrahydro-2H-pyran-2-carboxamido)propanoic acid
YRXSR

SEQ ID NO: 17 - protein, 5 aa, synthetic construct
  REGION 1..5: note = Synthetic Polypeptide
  SITE 3: note = 2-amino-3-((2S,3R,4S,5R,6S)-3,4,5,6-tetrahydroxytetrahydro-2H-pyran-2-carboxamido)propanoic acid
YRXRS

SEQ ID NO: 18 - protein, 5 aa, synthetic construct
  REGION 1..5: note = Synthetic Polypeptide
  SITE 3: note = 2-amino-3-((2S,3R,4S,5R,6S)-3,4,5,6-tetrahydroxytetrahydro-2H-pyran-2-carboxamido)propanoic acid
SRXRR

SEQ ID NO: 19-26 - skipped (8 entries)

SEQ ID NO: 27 - protein, 5 aa, synthetic construct
  REGION 1..5: note = Synthetic Polypeptide
  SITE 3: note = 2-amino-3-((2S,3R,4S,5R,6S)-3,4,5,6-tetrahydroxytetrahydro-2H-pyran-2-carboxamido)propanoic acid
ERXRR

SEQ ID NO: 28 - protein, 4 aa, synthetic construct
  REGION 1..4: note = Synthetic Polypeptide
SSSS

SEQ ID NO: 29 - skipped

SEQ ID NO: 30 - protein, 6 aa, synthetic construct
  REGION 1..6: note = Synthetic Polypeptide
  SITE 3: note = 2,2',2''-(10-(2-((5,6-diamino-6-oxohexyl)amino)-2-oxoethyl)-1,4,7,10-tetraazacyclododecane-1,4,7-triyl)triacetic acid
  MOD_RES 5: note = Glutamic Acid in position number 5 is linked to N6-(5-((3aR,4R,6aS)-2-oxohexahydro-1H-thieno[3,4-d]imidazol-4-yl)pentanoyl)-L-lysine in number position 6 through (PEG1)2
SEXEEX

SEQ ID NO: 31 - protein, 6 aa, synthetic construct
  REGION 1..6: note = Synthetic Polypeptide
  SITE 3: note = 2,2',2''-(10-(2-((5,6-diamino-6-oxohexyl)amino)-2-oxoethyl)-1,4,7,10-tetraazacyclododecane-1,4,7-triyl)triacetic acid
  SITE 6: note = 5-((6-(4-(2-amino-2-carboxyethyl)-1H-1,2,3-triazol-1-yl)hexyl)carbamoyl)-2-(6-amino-3-imino-4,5-disulfo-3H-xanthen-9-yl)benzoic acid
SEXEEX

SEQ ID NO: 32 - skipped

SEQ ID NO: 33 - protein, 6 aa, synthetic construct
  REGION 1..6: note = Synthetic Polypeptide
  SITE 3: note = 2,2',2''-(10-(2-((2-amino-2-carboxyethyl)amino)-2-oxoethyl)-1,4,7,10-tetraazacyclododecane-1,4,7-triyl)triacetic acid
  SITE 6: note = 5-((6-(4-(2-amino-2-carboxyethyl)-1H-1,2,3-triazol-1-yl)hexyl)carbamoyl)-2-(6-amino-3-imino-4,5-disulfo-3H-xanthen-9-yl)benzoic acid
SEXEEX

SEQ ID NO: 34 - skipped

SEQ ID NO: 35 - protein, 7 aa, synthetic construct
  REGION 1..7: note = Synthetic Polypeptide
  SITE 3: note = 2,2',2''-(10-(2-((2-amino-2-carboxyethyl)amino)-2-oxoethyl)-1,4,7,10-tetraazacyclododecane-1,4,7-triyl)triacetic acid
  SITE 6: note = 3-((2-((2-amino-2-carboxyethyl)amino)-2-oxoethyl)(metheyliumyl)(methyl)-lambda4-azaneyl)propane-1-sulfonate
  SITE 7: note = 5-((6-(4-(2-amino-2-carboxyethyl)-1H-1,2,3-triazol-1-yl)hexyl)carbamoyl)-2-(6-amino-3-imino-4,5-disulfo-3H-xanthen-9-yl)benzoic acid
SEXEEXX

SEQ ID NO: 36 - protein, 9 aa, synthetic construct
  REGION 1..9: note = Synthetic Polypeptide
  SITE 2: note = gamma-carboxyglutamic acid
  SITE 3: note = 5-((6-(4-(2-amino-2-carboxyethyl)-1H-1,2,3-triazol-1-yl)hexyl)carbamoyl)-2-(6-amino-3-imino-4,5-disulfo-3H-xanthen-9-yl)benzoic acid
EXXGVPTLQ

SEQ ID NO: 37 - protein, 9 aa, synthetic construct
  REGION 1..9: note = Synthetic Polypeptide
  SITE 2: note = gamma-carboxyglutamic acid
  SITE 3: note = 5-((6-(4-(2-amino-2-carboxyethyl)-1H-1,2,3-triazol-1-yl)hexyl)carbamoyl)-2-(6-amino-3-imino-4,5-disulfo-3H-xanthen-9-yl)benzoic acid
EXXEGRGDK

SEQ ID NO: 38 - protein, 8 aa, synthetic construct
  REGION 1..8: note = Synthetic Polypeptide
  SITE 2: note = gamma-carboxyglutamic acid
  SITE 3: note = 5-((6-(4-(2-amino-2-carboxyethyl)-1H-1,2,3-triazol-1-yl)hexyl)carbamoyl)-2-(6-amino-3-imino-4,5-disulfo-3H-xanthen-9-yl)benzoic acid
EXXKLPVM

SEQ ID NO: 39 - protein, 10 aa, synthetic construct
  REGION 1..10: note = Synthetic Polypeptide
  SITE 2: note = gamma-carboxyglutamic acid
  SITE 3: note = 5-((6-(4-(2-amino-2-carboxyethyl)-1H-1,2,3-triazol-1-yl)hexyl)carbamoyl)-2-(6-amino-3-imino-4,5-disulfo-3H-xanthen-9-yl)benzoic acid
EXXEGKLPVM

SEQ ID NO: 40-48 - skipped (9 entries)

SEQ ID NO: 49 - protein, 9 aa, synthetic construct
  REGION 1..9: note = Synthetic Polypeptide
  SITE 2: note = gamma-carboxyglutamic acid
  SITE 3: note = 1-(6-((3-(4-(2-amino-2-carboxyethyl)-1H-1,2,3-triazol-1-yl)propyl)amino)-6-oxohexyl)-3,3-dimethyl-2-((1E,3E)-5-((E)-1,3,3-trimethyl-5-sulfoindolin-2-ylidene)penta-1,3-dien-1-yl)-3H-indol-1-ium-5-sulfonate
SXXEERGDK

SEQ ID NO: 50 - protein, 9 aa, synthetic construct
  REGION 1..9: note = Synthetic Polypeptide
  SITE 2: note = gamma-carboxyglutamic acid
  SITE 3: note = 1-(6-((3-(4-(2-amino-2-carboxyethyl)-1H-1,2,3-triazol-1-yl)propyl)amino)-6-oxohexyl)-3,3-dimethyl-2-((1E,3E)-5-((E)-1,3,3-trimethyl-5-sulfoindolin-2-ylidene)penta-1,3-dien-1-yl)-3H-indol-1-ium-5-sulfonate
EXXGVPTLQ

SEQ ID NO: 51 - protein, 9 aa, synthetic construct
  REGION 1..9: note = Synthetic Polypeptide
  SITE 2: note = gamma-carboxyglutamic acid
  SITE 3: note = 1-(6-((3-(4-(2-amino-2-carboxyethyl)-1H-1,2,3-triazol-1-yl)propyl)amino)-6-oxohexyl)-3,3-dimethyl-2-((1E,3E)-5-((E)-1,3,3-trimethyl-5-sulfoindolin-2-ylidene)penta-1,3-dien-1-yl)-3H-indol-1-ium-5-sulfonate
EXXEGRGDK

SEQ ID NO: 52 - protein, 8 aa, synthetic construct
  REGION 1..8: note = Synthetic Polypeptide
  SITE 2: note = gamma-carboxyglutamic acid
  SITE 3: note = 1-(6-((3-(4-(2-amino-2-carboxyethyl)-1H-1,2,3-triazol-1-yl)propyl)amino)-6-oxohexyl)-3,3-dimethyl-2-((1E,3E)-5-((E)-1,3,3-trimethyl-5-sulfoindolin-2-ylidene)penta-1,3-dien-1-yl)-3H-indol-1-ium-5-sulfonate
EXXKLPVM

SEQ ID NO: 53 - protein, 10 aa, synthetic construct
  REGION 1..10: note = Synthetic Polypeptide
  SITE 2: note = gamma-carboxyglutamic acid
  SITE 3: note = 1-(6-((3-(4-(2-amino-2-carboxyethyl)-1H-1,2,3-triazol-1-yl)propyl)amino)-6-oxohexyl)-3,3-dimethyl-2-((1E,3E)-5-((E)-1,3,3-trimethyl-5-sulfoindolin-2-ylidene)penta-1,3-dien-1-yl)-3H-indol-1-ium-5-sulfonate
EXXEGKLPVM

SEQ ID NO: 54 - protein, 6 aa, synthetic construct
  REGION 1..6: note = Synthetic Polypeptide
  SITE 4: note = 1-(6-((3-(4-(2-amino-2-carboxyethyl)-1H-1,2,3-triazol-1-yl)propyl)amino)-6-oxohexyl)-3,3-dimethyl-2-((1E,3E)-5-((E)-1,3,3-trimethyl-5-sulfoindolin-2-ylidene)penta-1,3-dien-1-yl)-3H-indol-1-ium-5-sulfonate
  SITE 6: note = 3-((2-((2-amino-2-carboxyethyl)amino)-2-oxoethyl)(metheyliumyl)(methyl)-lambda4-azaneyl)propane-1-sulfonate
SEEXEX

SEQ ID NO: 55 - protein, 7 aa, synthetic construct
  REGION 1..7: note = Synthetic Polypeptide
  SITE 4: note = 1-(6-((3-(4-(2-amino-2-carboxyethyl)-1H-1,2,3-triazol-1-yl)propyl)amino)-6-oxohexyl)-3,3-dimethyl-2-((1E,3E)-5-((E)-1,3,3-trimethyl-5-sulfoindolin-2-ylidene)penta-1,3-dien-1-yl)-3H-indol-1-ium-5-sulfonate
  SITE 6: note = 3-((2-((2-amino-2-carboxyethyl)amino)-2-oxoethyl)(metheyliumyl)(methyl)-lambda4-azaneyl)propane-1-sulfonate
  MOD_RES 7: note = N6-(4-(4-iodophenyl)butanoyl)-lysine
SEEXEXX

SEQ ID NO: 56 - protein, 5 aa, synthetic construct
  REGION 1..5: note = Synthetic Polypeptide
  SITE 4: note = 1-(6-((3-(4-(2-amino-2-carboxyethyl)-1H-1,2,3-triazol-1-yl)propyl)amino)-6-oxohexyl)-3,3-dimethyl-2-((1E,3E)-5-((E)-1,3,3-trimethyl-5-sulfoindolin-2-ylidene)penta-1,3-dien-1-yl)-3H-indol-1-ium-5-sulfonate
SEEXE

SEQ ID NO: 57 - protein, 6 aa, synthetic construct
  REGION 1..6: note = Synthetic Polypeptide
  SITE 4: note = 2,2',2''-(10-(2-((5,6-diamino-6-oxohexyl)amino)-2-oxoethyl)-1,4,7,10-tetraazacyclododecane-1,4,7-triyl)triacetic acid
  SITE 6: note = 3-((2-((2-amino-2-carboxyethyl)amino)-2-oxoethyl)(metheyliumyl)(methyl)-lambda4-azaneyl)propane-1-sulfonate
SEEXEX

SEQ ID NO: 58 - protein, 7 aa, synthetic construct
  REGION 1..7: note = Synthetic Polypeptide
  SITE 4: note = 2,2',2''-(10-(2-((2-amino-2-carboxyethyl)amino)-2-oxoethyl)-1,4,7,10-tetraazacyclododecane-1,4,7-triyl)triacetic acid
  SITE 6: note = 3-((2-((2-amino-2-carboxyethyl)amino)-2-oxoethyl)(metheyliumyl)(methyl)- lambda4-azaneyl)propane-1-sulfonate
  MOD_RES 7: note = N6-(4-(4-iodophenyl)butanoyl)-lysine
SEEXEXX

SEQ ID NO: 59 - protein, 5 aa, synthetic construct
  REGION 1..5: note = Synthetic Polypeptide
  SITE 4: note = 2,2',2''-(10-(2-((2-amino-2-carboxyethyl)amino)-2-oxoethyl)-1,4,7,10-tetraazacyclododecane-1,4,7-triyl)triacetic acid
SEEXE

SEQ ID NO: 60 - skipped

SEQ ID NO: 61 - protein, 6 aa, synthetic construct
  REGION 1..6: note = Synthetic Polypeptide
  SITE 4: note = 1-(6-((3-(4-(2-amino-2-carboxyethyl)-1H-1,2,3-triazol-1-yl)propyl)amino)-6-oxohexyl)-3,3-dimethyl-2-((1E,3E)-5-((E)-1,3,3-trimethyl-5-sulfoindolin-2-ylidene)penta-1,3-dien-1-yl)-3H-indol-1-ium-5-sulfonate
  MOD_RES 6: note = N6-(2-(4-iodophenyl)acetyl)-D-lysine
SEEXEX

SEQ ID NO: 62-66 - skipped (5 entries)

SEQ ID NO: 67 - protein, 7 aa, synthetic construct
  REGION 1..7: note = Synthetic Polypeptide
  SITE 4: note = 1-(6-((3-(4-(2-amino-2-carboxyethyl)-1H-1,2,3-triazol-1-yl)propyl)amino)-6-oxohexyl)-3,3-dimethyl-2-((1E,3E)-5-((E)-1,3,3-trimethyl-5-sulfoindolin-2-ylidene)penta-1,3-dien-1-yl)-3H-indol-1-ium-5-sulfonate
  SITE 5: note = 3-((2-((2-amino-2-carboxyethyl)amino)-2-oxoethyl)(metheyliumyl)(methyl)- lambda4-azaneyl)propane-1-sulfonate
  MOD_RES 6: note = N6-(2-(4-iodophenyl)acetyl)-D-lysine
SEEXEXX

SEQ ID NO: 68 - skipped

SEQ ID NO: 69 - protein, 6 aa, synthetic construct
  REGION 1..6: note = Synthetic Polypeptide
  SITE 4: note = 1-(6-((3-(4-(2-amino-2-carboxyethyl)-1H-1,2,3-triazol-1-yl)propyl)amino)-6-oxohexyl)-3,3-dimethyl-2-((1E,3E)-5-((E)-1,3,3-trimethyl-5-sulfoindolin-2-ylidene)penta-1,3-dien-1-yl)-3H-indol-1-ium-5-sulfonate
  SITE 6: note = Trityl resin binds to the C-terminus of N6-(2-(4-iodophenyl)acetyl)-D-lysine to produce the C-terminus, which is -COOH.
  MOD_RES 6: note = N6-(2-(4-iodophenyl)acetyl)-D-lysine
SEEXEX

SEQ ID NO: 70 - protein, 5 aa, synthetic construct
  REGION 1..5: note = Synthetic Polypeptide
  SITE 4: note = 1-(6-((3-(4-(2-amino-2-carboxyethyl)-1H-1,2,3-triazol-1-yl)propyl)amino)-6-oxohexyl)-3,3-dimethyl-2-((1E,3E)-5-((E)-1,3,3-trimethyl-5-sulfoindolin-2-ylidene)penta-1,3-dien-1-yl)-3H-indol-1-ium-5-sulfonate
SSEXE

SEQ ID NO: 71 - protein, 5 aa, synthetic construct
  REGION 1..5: note = Synthetic Polypeptide
  SITE 4: note = (R)-2,2'-(4-(2-((2-amino-2-carboxyethyl)amino)-2-oxoethyl)-10-(2-amino-2-oxoethyl)-1,4,7,10-tetraazacyclododecane-1,7-diyl)diacetic acid
SEEXE

SEQ ID NO: 72 - protein, 5 aa, synthetic construct
  REGION 1..5: note = Synthetic Polypeptide
  SITE 4: note = (2R)-2-amino-3-(3-(4-((1,4,7,10-tetrakis(2-amino-2-oxoethyl)-1,4,7,10-tetraazacyclododecan-2-yl)methyl)phenyl)thioureido)propanoic acid
SEEXE

SEQ ID NO: 73 - protein, 9 aa, synthetic construct
  REGION 1..9: note = Synthetic Polypeptide
  SITE 1: note = (R)-2-amino-6-(4-(4-sulfamoylphenyl)-1H-1,2,3-triazol-1-yl)hexanoic acid
  SITE 7: note = (R)-2-amino-4-(4-(4-sulfamoylphenyl)-1H-1,2,3-triazol-1-yl)butanoic acid
  SITE 9: note = (R)-2-amino-4-(4-(4-sulfamoylphenyl)-1H-1,2,3-triazol-1-yl)butanoic acid; note = (R)-2-amino-4-(4-(4-sulfamoylphenyl)-1H-1,2,3-triazol-1-yl)butanoic acid is linked via an amide linkage to the carboxyl group of side chain in the Glutamic Acid at position 8 .
  REGION 1..8: note = (R)-2-amino-6-(4-(4-sulfamoylphenyl)-1H-1,2,3-triazol-1-yl)hexanoic acid at position 1 and Glutamic Acid at position 8 are linked via an amide linkage to form a cyclic peptide.
  SITE 9: note = The (R)-2-amino-4-(4-(4-sulfamoylphenyl)-1H-1,2,3-triazol-1-yl)butanoic acid in position number 9 is linked via an amide linkage to another sequence.
XYRFRRXEX

SEQ ID NO: 74 - protein, 8 aa, synthetic construct
  REGION 1..8: note = Synthetic Polypeptide
  REGION 1..8: note = (R)-2-amino-6-(4-(4-sulfamoylphenyl)-1H-1,2,3-triazol-1-yl)hexanoic acid at position 1 and Glutamic Acid at position 8 are linked via an amide linkage to form a cyclic peptide.
  SITE 1: note = (R)-2-amino-6-(4-(4-sulfamoylphenyl)-1H-1,2,3-triazol-1-yl)hexanoic acid
  SITE 2: note = (R)-2-amino-4-(4-(4-sulfamoylphenyl)-1H-1,2,3-triazol-1-yl)butanoic acid
  SITE 7: note = (R)-2-amino-4-(4-(4-sulfamoylphenyl)-1H-1,2,3-triazol-1-yl)butanoic acid
  SITE 8: note = The side chain of the glutamic acid in position number 8 is linked via an amide linkage to another sequence.
XXRFRRXE

SEQ ID NO: 75 - protein, 8 aa, synthetic construct
  REGION 1..8: note = Synthetic Polypeptide
  REGION 1..8: note = (R)-2-amino-6-(4-(4-sulfamoylphenyl)-1H-1,2,3-triazol-1-yl)hexanoic acid at position 1 and Glutamic Acid at position 8 are linked via an amide linkage to form a cyclic peptide.
  SITE 1: note = (R)-2-amino-6-(4-(4-sulfamoylphenyl)-1H-1,2,3-triazol-1-yl)hexanoic acid
  SITE 2: note = (R)-2-amino-4-(4-(4-sulfamoylphenyl)-1H-1,2,3-triazol-1-yl)butanoic acid
  SITE 7: note = (R)-2-amino-4-(4-(4-sulfamoylphenyl)-1H-1,2,3-triazol-1-yl)butanoic acid
  SITE 8: note = The side chain of the glutamic acid in position number 8 is linked via an amide linkage to another sequence.
XXRARRXE

SEQ ID NO: 76 - protein, 8 aa, synthetic construct
  REGION 1..8: note = Synthetic Polypeptide
  REGION 1..8: note = (R)-2-amino-4-(4-(4-sulfamoylphenyl)-1H-1,2,3-triazol-1-yl)butanoic acid at position 1 and Glutamic Acid at position 8 are linked via an amide linkage to form a cyclic peptide.
  SITE 1: note = (R)-2-amino-4-(4-(4-sulfamoylphenyl)-1H-1,2,3-triazol-1-yl)butanoic acid
  SITE 2: note = (R)-2-amino-4-(4-(4-sulfamoylphenyl)-1H-1,2,3-triazol-1-yl)butanoic acid
  SITE 7: note = (R)-2-amino-4-(4-(4-sulfamoylphenyl)-1H-1,2,3-triazol-1-yl)butanoic acid
  SITE 8: note = The side chain of the glutamic acid in position number 8 is linked via an amide linkage to another sequence.
XXRARRXE

SEQ ID NO: 77 - protein, 9 aa, synthetic construct
  REGION 1..9: note = Synthetic Polypeptide
  REGION 1..8: note = (R)-2-amino-4-(4-(4-sulfamoylphenyl)-1H-1,2,3-triazol-1-yl)butanoic acid at position 1 and Glutamic Acid at position 8 are linked via an amide linkage to form a cyclic peptide.
  SITE 1: note = (R)-2-amino-4-(4-(4-sulfamoylphenyl)-1H-1,2,3-triazol-1-yl)butanoic acid
  SITE 7: note = (R)-2-amino-4-(4-(4-sulfamoylphenyl)-1H-1,2,3-triazol-1-yl)butanoic acid
  SITE 9: note = (R)-2-amino-4-(4-(4-sulfamoylphenyl)-1H-1,2,3-triazol-1-yl)butanoic acid is linked via an amide linkage to the carboxyl group of side chain in the Glutamic Acid at position 8.; note = (R)-2-amino-4-(4-(4-sulfamoylphenyl)-1H-1,2,3-triazol-1-yl)butanoic acid
  SITE 9: note = The (R)-2-amino-4-(4-(4-sulfamoylphenyl)-1H-1,2,3-triazol-1-yl)butanoic acid in position number 9 is linked via an amide linkage to another sequence.
XYRFRRXEX

SEQ ID NO: 78 - protein, 9 aa, synthetic construct
  REGION 1..9: note = Synthetic Polypeptide
  REGION 1..8: note = (R)-2-amino-6-(4-(4-sulfamoylphenyl)-1H-1,2,3-triazol-1-yl)hexanoic acid at position 1 and Glutamic Acid at position 8 are linked via an amide linkage to form a cyclic peptide.
  SITE 1: note = (R)-2-amino-6-(4-(4-sulfamoylphenyl)-1H-1,2,3-triazol-1-yl)hexanoic acid
  SITE 7: note = (R)-2-amino-4-(4-(4-sulfamoylphenyl)-1H-1,2,3-triazol-1-yl)butanoic acid
  SITE 9: note = (R)-2-amino-4-(4-(4-sulfamoylphenyl)-1H-1,2,3-triazol-1-yl)butanoic acid is linked via an amide linkage to the carboxyl group of side chain in the Glutamic Acid at position 8.; note = (R)-2-amino-4-(4-(4-sulfamoylphenyl)-1H-1,2,3-triazol-1-yl)butanoic acid
  SITE 9: note = The (R)-2-amino-4-(4-(4-sulfamoylphenyl)-1H-1,2,3-triazol-1-yl)butanoic acid in position number 9 is linked via an amide linkage to another sequence.
XYRARRXEX

SEQ ID NO: 79 - protein, 9 aa, synthetic construct
  REGION 1..9: note = Synthetic Polypeptide
  REGION 1..8: note = (R)-2-amino-6-(4-(4-sulfamoylphenyl)-1H-1,2,3-triazol-1-yl)hexanoic acid at position 1 and Glutamic Acid at position 8 are linked via an amide linkage to form a cyclic peptide.
  SITE 1: note = (R)-2-amino-6-(4-(4-sulfamoylphenyl)-1H-1,2,3-triazol-1-yl)hexanoic acid
  SITE 7: note = (R)-2-amino-4-(4-(4-sulfamoylphenyl)-1H-1,2,3-triazol-1-yl)butanoic acid
  SITE 9: note = (R)-2-amino-4-(4-(4-sulfamoylphenyl)-1H-1,2,3-triazol-1-yl)butanoic acid is linked via an amide linkage to the carboxyl group of side chain in the Glutamic Acid at position 8.; note = (R)-2-amino-4-(4-(4-sulfamoylphenyl)-1H-1,2,3-triazol-1-yl)butanoic acid
  SITE 9: note = The (R)-2-amino-4-(4-(4-sulfamoylphenyl)-1H-1,2,3-triazol-1-yl)butanoic acid in position number 9 is linked via an amide linkage to another sequence.
XARFRRXEX

SEQ ID NO: 80 - protein, 8 aa, synthetic construct
  REGION 1..8: note = Synthetic Polypeptide
  REGION 1..7: note = (R)-2-amino-6-(4-(4-sulfamoylphenyl)-1H-1,2,3-triazol-1-yl)hexanoic acid at position 1 and Glutamic Acid at position 7 are linked via an amide linkage to form a cyclic peptide.
  SITE 1: note = (R)-2-amino-6-(4-(4-sulfamoylphenyl)-1H-1,2,3-triazol-1-yl)hexanoic acid
  SITE 6: note = (R)-2-amino-4-(4-(4-sulfamoylphenyl)-1H-1,2,3-triazol-1-yl)butanoic acid
  SITE 8: note = (R)-2-amino-4-(4-(4-sulfamoylphenyl)-1H-1,2,3-triazol-1-yl)butanoic acid; note = (R)-2-amino-4-(4-(4-sulfamoylphenyl)-1H-1,2,3-triazol-1-yl)butanoic acid is linked via an amide linkage to the carboxyl group of side chain in the Glutamic Acid at position 7.
  SITE 8: note = The (R)-2-amino-4-(4-(4-sulfamoylphenyl)-1H-1,2,3-triazol-1-yl)butanoic acid in position number 8 is linked via an amide linkage to another sequence.
XRFRRXEX

SEQ ID NO: 81 - protein, 9 aa, synthetic construct
  REGION 1..9: note = Synthetic Polypeptide
  REGION 1..8: note = (R)-2-amino-6-(4-(4-sulfamoylphenyl)-1H-1,2,3-triazol-1-yl)hexanoic acid at position 1 and Glutamic Acid at position 8 are linked via an amide linkage to form a cyclic peptide.
  SITE 1: note = (R)-2-amino-6-(4-(4-sulfamoylphenyl)-1H-1,2,3-triazol-1-yl)hexanoic acid
  SITE 7: note = (R)-2-amino-4-(4-(4-sulfamoylphenyl)-1H-1,2,3-triazol-1-yl)butanoic acid
  SITE 9: note = (R)-2-amino-4-(4-(4-sulfamoylphenyl)-1H-1,2,3-triazol-1-yl)butanoic acid; note = (R)-2-amino-4-(4-(4-sulfamoylphenyl)-1H-1,2,3-triazol-1-yl)butanoic acid is linked via an amide linkage to the carboxyl group of side chain in the Glutamic Acid at position 8.
  SITE 9: note = The (R)-2-amino-4-(4-(4-sulfamoylphenyl)-1H-1,2,3-triazol-1-yl)butanoic acid in position number 9 is linked via an amide linkage to another sequence.
XARARRXEX

SEQ ID NO: 82 - protein, 8 aa, synthetic construct
  REGION 1..8: note = Synthetic Polypeptide
  REGION 1..7: note = (R)-2-amino-6-(4-(4-sulfamoylphenyl)-1H-1,2,3-triazol-1-yl)hexanoic acid at position 1 and Glutamic Acid at position 7 are linked via an amide linkage to form a cyclic peptide.
  SITE 1: note = (R)-2-amino-6-(4-(4-sulfamoylphenyl)-1H-1,2,3-triazol-1-yl)hexanoic acid
  SITE 6: note = (R)-2-amino-4-(4-(4-sulfamoylphenyl)-1H-1,2,3-triazol-1-yl)butanoic acid
  SITE 8: note = (R)-2-amino-4-(4-(4-sulfamoylphenyl)-1H-1,2,3-triazol-1-yl)butanoic acid is linked via an amide linkage to the carboxyl group of side chain in the Glutamic Acid at position 7.; note = (R)-2-amino-4-(4-(4-sulfamoylphenyl)-1H-1,2,3-triazol-1-yl)butanoic acid
  SITE 8: note = The (R)-2-amino-4-(4-(4-sulfamoylphenyl)-1H-1,2,3-triazol-1-yl)butanoic acid in position number 8 is linked via an amide linkage to another sequence.
XRARRXEX

SEQ ID NO: 83 - protein, 8 aa, synthetic construct
  REGION 1..8: note = Synthetic Polypeptide
  REGION 1..8: note = (R)-2-amino-6-(4-(4-sulfamoylphenyl)-1H-1,2,3-triazol-1-yl)hexanoic acid at position 1 and Glutamic Acid at position 8 are linked via an amide linkage to form a cyclic peptide.
  SITE 1: note = (R)-2-amino-6-(4-(4-sulfamoylphenyl)-1H-1,2,3-triazol-1-yl)hexanoic acid
  SITE 2: note = (R)-2-amino-4-(4-(4-sulfamoylphenyl)-1H-1,2,3-triazol-1-yl)butanoic acid
  SITE 4: note = 2-amino-3-((2S,3R,4S,5R,6S)-3,4,5,6-tetrahydroxytetrahydro-2H-pyran-2-carboxamido)propanoic acid
  SITE 7: note = (R)-2-amino-4-(4-(4-sulfamoylphenyl)-1H-1,2,3-triazol-1-yl)butanoic acid
  SITE 8: note = The side chain of the glutamic acid in position number 8 is linked via an amide linkage to another sequence.
XXRXRRXE

SEQ ID NO: 84 - protein, 8 aa, synthetic construct
  REGION 1..8: note = (R)-2-amino-6-(4-(4-sulfamoylphenyl)-1H-1,2,3-triazol-1-yl)hexanoic acid at position 1 and Glutamic Acid at position 8 are linked via an amide linkage to form a cyclic peptide.; note = Synthetic Polypeptide
  SITE 1: note = (R)-2-amino-6-(4-(4-sulfamoylphenyl)-1H-1,2,3-triazol-1-yl)hexanoic acid
  SITE 2: note = (R)-2-amino-4-(4-(4-sulfamoylphenyl)-1H-1,2,3-triazol-1-yl)butanoic acid
  MOD_RES 4: note = N6-(4-(4-iodophenyl)butanoyl)-lysine
  SITE 7: note = (R)-2-amino-4-(4-(4-sulfamoylphenyl)-1H-1,2,3-triazol-1-yl)butanoic acid
  SITE 8: note = The side chain of the glutamic acid in position number 8 is linked via an amide linkage to another sequence.
XXRXRRXE

SEQ ID NO: 85 - protein, 8 aa, synthetic construct
  REGION 1..8: note = Synthetic Polypeptide; note = (R)-2-amino-6-(4-(4-sulfamoylphenyl)-1H-1,2,3-triazol-1-yl)hexanoic acid at position 1 and Glutamic Acid at position 8 are linked via an amide linkage to form a cyclic peptide.
  SITE 1: note = (R)-2-amino-6-(4-(4-sulfamoylphenyl)-1H-1,2,3-triazol-1-yl)hexanoic acid
  SITE 2: note = (R)-2-amino-4-(4-(4-sulfamoylphenyl)-1H-1,2,3-triazol-1-yl)butanoic acid
  SITE 7: note = (R)-2-amino-4-(4-(4-sulfamoylphenyl)-1H-1,2,3-triazol-1-yl)butanoic acid
  SITE 8: note = The side chain of the glutamic acid in position number 8 is linked via an amide linkage to another sequence.
XXRNRRXE

SEQ ID NO: 86 - protein, 8 aa, synthetic construct
  REGION 1..8: note = Synthetic Polypeptide; note = (R)-2-amino-6-(4-(4-sulfamoylphenyl)-1H-1,2,3-triazol-1-yl)hexanoic acid at position 1 and Glutamic Acid at position 8 are linked via an amide linkage to form a cyclic peptide.
  SITE 1: note = (R)-2-amino-6-(4-(4-sulfamoylphenyl)-1H-1,2,3-triazol-1-yl)hexanoic acid
  SITE 2: note = (R)-2-amino-4-(4-(4-sulfamoylphenyl)-1H-1,2,3-triazol-1-yl)butanoic acid
  SITE 7: note = (R)-2-amino-4-(4-(4-sulfamoylphenyl)-1H-1,2,3-triazol-1-yl)butanoic acid
  SITE 8: note = The side chain of the glutamic acid in position number 8 is linked via an amide linkage to another sequence.
XXAAAAXE

SEQ ID NO: 87 - protein, 8 aa, synthetic construct
  REGION 1..8: note = Synthetic Polypeptide; note = (R)-2-amino-6-(4-(4-sulfamoylphenyl)-1H-1,2,3-triazol-1-yl)hexanoic acid at position 1 and Glutamic Acid at position 8 are linked via an amide linkage to form a cyclic peptide.
  SITE 1: note = (R)-2-amino-6-(4-(4-sulfamoylphenyl)-1H-1,2,3-triazol-1-yl)hexanoic acid
  SITE 2: note = (R)-2-amino-4-(4-(4-sulfamoylphenyl)-1H-1,2,3-triazol-1-yl)butanoic acid
  SITE 7: note = (R)-2-amino-4-(4-(4-sulfamoylphenyl)-1H-1,2,3-triazol-1-yl)butanoic acid
  SITE 8: note = The side chain of the glutamic acid in position number 8 is linked via an amide linkage to another sequence.
XXRERRXE

SEQ ID NO: 88 - protein, 8 aa, synthetic construct
  REGION 1..8: note = Synthetic Polypeptide; note = (R)-2-amino-6-(4-(4-sulfamoylphenyl)-1H-1,2,3-triazol-1-yl)hexanoic acid at position 1 and Glutamic Acid at position 8 are linked via an amide linkage to form a cyclic peptide.
  SITE 1: note = (R)-2-amino-6-(4-(4-sulfamoylphenyl)-1H-1,2,3-triazol-1-yl)hexanoic acid
  SITE 7: note = (R)-2-amino-4-(4-(4-sulfamoylphenyl)-1H-1,2,3-triazol-1-yl)butanoic acid
  SITE 8: note = The side chain of the glutamic acid in position number 8 is linked via an amide linkage to another sequence.
XYRFRRXE

SEQ ID NO: 89 - protein, 8 aa, synthetic construct
  REGION 1..8: note = (R)-2-amino-6-(4-(4-sulfamoylphenyl)-1H-1,2,3-triazol-1-yl)hexanoic acid at position 1 and Glutamic Acid at position 8 are linked via an amide linkage to form a cyclic peptide.; note = Synthetic Polypeptide
  SITE 1: note = (R)-2-amino-6-(4-(4-sulfamoylphenyl)-1H-1,2,3-triazol-1-yl)hexanoic acid
  SITE 7: note = (R)-2-amino-6-(4-(4-sulfamoylphenyl)-1H-1,2,3-triazol-1-yl)hexanoic acid
  SITE 8: note = The side chain of the glutamic acid in position number 8 is linked via an amide linkage to another sequence.
XYRFRRXE

SEQ ID NO: 90 - protein, 9 aa, synthetic construct
  REGION 1..9: note = Synthetic Polypeptide
  REGION 1..8: note = (R)-2-amino-6-(4-(4-sulfamoylphenyl)-1H-1,2,3-triazol-1-yl)hexanoic acid at position 1 and Glutamic Acid at position 8 are linked via an amide linkage to form a cyclic peptide.
  SITE 1: note = (R)-2-amino-6-(4-(4-sulfamoylphenyl)-1H-1,2,3-triazol-1-yl)hexanoic acid
  SITE 4: note = 2-amino-3-((2S,3R,4S,5R,6S)-3,4,5,6-tetrahydroxytetrahydro-2H-pyran-2-carboxamido)propanoic acid
  SITE 7: note = (R)-2-amino-4-(4-(4-sulfamoylphenyl)-1H-1,2,3-triazol-1-yl)butanoic acid
  SITE 9: note = (R)-2-amino-4-(4-(4-sulfamoylphenyl)-1H-1,2,3-triazol-1-yl)butanoic acid is linked via an amide linkage to the carboxyl group of side chain in the Glutamic Acid at position 8.; note = (R)-2-amino-4-(4-(4-sulfamoylphenyl)-1H-1,2,3-triazol-1-yl)butanoic acid
  SITE 9: note = The (R)-2-amino-4-(4-(4-sulfamoylphenyl)-1H-1,2,3-triazol-1-yl)butanoic acid in position number 9 is linked via an amide linkage to another sequence.
XYRXRRXEX

SEQ ID NO: 91-92 - skipped (2 entries)

SEQ ID NO: 93 - protein, 9 aa, synthetic construct
  REGION 1..9: note = Synthetic Polypeptide
  REGION 1..8: note = (R)-2-amino-6-(4-(4-sulfamoylphenyl)-1H-1,2,3-triazol-1-yl)hexanoic acid at position 1 and Glutamic Acid at position 8 are linked via an amide linkage to form a cyclic peptide.
  SITE 1: note = (R)-2-amino-6-(4-(4-sulfamoylphenyl)-1H-1,2,3-triazol-1-yl)hexanoic acid
  SITE 4: note = 2-amino-3-((2S,3R,4S,5R,6S)-3,4,5,6-tetrahydroxytetrahydro-2H-pyran-2-carboxamido)propanoic acid
  SITE 7: note = (R)-2-amino-4-(4-(4-sulfamoylphenyl)-1H-1,2,3-triazol-1-yl)butanoic acid
  SITE 9: note = (R)-2-amino-4-(4-(4-sulfamoylphenyl)-1H-1,2,3-triazol-1-yl)butanoic acid; note = (R)-2-amino-4-(4-(4-sulfamoylphenyl)-1H-1,2,3-triazol-1-yl)butanoic acid is linked via an amide linkage to the carboxyl group of side chain in the Glutamic Acid at position 8.
  SITE 9: note = The (R)-2-amino-4-(4-(4-sulfamoylphenyl)-1H-1,2,3-triazol-1-yl)butanoic acid in position number 9 is linked via an amide linkage to another sequence.
XYSXRRXEX

SEQ ID NO: 94 - protein, 9 aa, synthetic construct
  REGION 1..9: note = Synthetic Polypeptide
  REGION 1..8: note = (R)-2-amino-6-(4-(4-sulfamoylphenyl)-1H-1,2,3-triazol-1-yl)hexanoic acid at position 1 and Glutamic Acid at position 8 are linked via an amide linkage to form a cyclic peptide.
  SITE 1: note = (R)-2-amino-6-(4-(4-sulfamoylphenyl)-1H-1,2,3-triazol-1-yl)hexanoic acid
  SITE 4: note = 2-amino-3-((2S,3R,4S,5R,6S)-3,4,5,6-tetrahydroxytetrahydro-2H-pyran-2-carboxamido)propanoic acid
  SITE 7: note = (R)-2-amino-4-(4-(4-sulfamoylphenyl)-1H-1,2,3-triazol-1-yl)butanoic acid
  SITE 9: note = (R)-2-amino-4-(4-(4-sulfamoylphenyl)-1H-1,2,3-triazol-1-yl)butanoic acid; note = (R)-2-amino-4-(4-(4-sulfamoylphenyl)-1H-1,2,3-triazol-1-yl)butanoic acid is linked via an amide linkage to the carboxyl group of side chain in the Glutamic Acid at position 8.
  SITE 9: note = The (R)-2-amino-4-(4-(4-sulfamoylphenyl)-1H-1,2,3-triazol-1-yl)butanoic acid in position number 9 is linked via an amide linkage to another sequence.
XYRXSRXEX

SEQ ID NO: 95 - protein, 9 aa, synthetic construct
  REGION 1..9: note = Synthetic Polypeptide
  REGION 1..8: note = (R)-2-amino-6-(4-(4-sulfamoylphenyl)-1H-1,2,3-triazol-1-yl)hexanoic acid at position 1 and Glutamic Acid at position 8 are linked via an amide linkage to form a cyclic peptide.
  SITE 1: note = (R)-2-amino-6-(4-(4-sulfamoylphenyl)-1H-1,2,3-triazol-1-yl)hexanoic acid
  SITE 4: note = 2-amino-3-((2S,3R,4S,5R,6S)-3,4,5,6-tetrahydroxytetrahydro-2H-pyran-2-carboxamido)propanoic acid
  SITE 7: note = (R)-2-amino-4-(4-(4-sulfamoylphenyl)-1H-1,2,3-triazol-1-yl)butanoic acid
  SITE 9: note = (R)-2-amino-4-(4-(4-sulfamoylphenyl)-1H-1,2,3-triazol-1-yl)butanoic acid is linked via an amide linkage to the carboxyl group of side chain in the Glutamic Acid at position 8.; note = (R)-2-amino-4-(4-(4-sulfamoylphenyl)-1H-1,2,3-triazol-1-yl)butanoic acid
  SITE 9: note = The (R)-2-amino-4-(4-(4-sulfamoylphenyl)-1H-1,2,3-triazol-1-yl)butanoic acid in position number 9 is linked via an amide linkage to another sequence.
XYRXRSXEX

SEQ ID NO: 96 - protein, 9 aa, synthetic construct
  REGION 1..9: note = (R)-2-amino-6-(4-(4-sulfamoylphenyl)-1H-1,2,3-triazol-1-yl)hexanoic acid
  REGION 1..8: note = (R)-2-amino-6-(4-(4-sulfamoylphenyl)-1H-1,2,3-triazol-1-yl)hexanoic acid at position 1 and Glutamic Acid at position 8 are linked via an amide linkage to form a cyclic peptide.
  SITE 1: note = (R)-2-amino-6-(4-(4-sulfamoylphenyl)-1H-1,2,3-triazol-1-yl)hexanoic acid
  SITE 4: note = 2-amino-3-((2S,3R,4S,5R,6S)-3,4,5,6-tetrahydroxytetrahydro-2H-pyran-2-carboxamido)propanoic acid
  SITE 7: note = (R)-2-amino-4-(4-(4-sulfamoylphenyl)-1H-1,2,3-triazol-1-yl)butanoic acid
  SITE 9: note = (R)-2-amino-4-(4-(4-sulfamoylphenyl)-1H-1,2,3-triazol-1-yl)butanoic acid; note = (R)-2-amino-4-(4-(4-sulfamoylphenyl)-1H-1,2,3-triazol-1-yl)butanoic acid is linked via an amide linkage to the carboxyl group of side chain in the Glutamic Acid at position 8.
  SITE 9: note = The (R)-2-amino-4-(4-(4-sulfamoylphenyl)-1H-1,2,3-triazol-1-yl)butanoic acid in position number 9 is linked via an amide linkage to another sequence.
XSRXRRXEX

SEQ ID NO: 97 - protein, 9 aa, synthetic construct
  REGION 1..8: note = (R)-2-amino-6-(4-(4-sulfamoylphenyl)-1H-1,2,3-triazol-1-yl)hexanoic acid at position 1 and Glutamic Acid at position 8 are linked via an amide linkage to form a cyclic peptide.
  REGION 1..9: note = Synthetic Polypeptide
  SITE 1: note = (R)-2-amino-6-(4-(4-sulfamoylphenyl)-1H-1,2,3-triazol-1-yl)hexanoic acid
  SITE 2: note = 2-amino-3-((2S,3R,4S,5R,6S)-3,4,5,6-tetrahydroxytetrahydro-2H-pyran-2-carboxamido)propanoic acid
  SITE 4: note = 2-amino-3-((2S,3R,4S,5R,6S)-3,4,5,6-tetrahydroxytetrahydro-2H-pyran-2-carboxamido)propanoic acid
  SITE 7: note = (R)-2-amino-4-(4-(4-sulfamoylphenyl)-1H-1,2,3-triazol-1-yl)butanoic acid
  SITE 9: note = (R)-2-amino-4-(4-(4-sulfamoylphenyl)-1H-1,2,3-triazol-1-yl)butanoic acid is linked via an amide linkage to the carboxyl group of side chain in the Glutamic Acid at position 8.; note = (R)-2-amino-4-(4-(4-sulfamoylphenyl)-1H-1,2,3-triazol-1-yl)butanoic acid
  SITE 9: note = The (R)-2-amino-4-(4-(4-sulfamoylphenyl)-1H-1,2,3-triazol-1-yl)butanoic acid in position number 9 is linked via an amide linkage to another sequence.
XXRXRRXEX

SEQ ID NO: 98 - protein, 9 aa, synthetic construct
  REGION 1..9: note = Synthetic Polypeptide
  REGION 1..8: note = (R)-2-amino-6-(4-(4-sulfamoylphenyl)-1H-1,2,3-triazol-1-yl)hexanoic acid at position 1 and Glutamic Acid at position 8 are linked via an amide linkage to form a cyclic peptide.
  SITE 1: note = (R)-2-amino-6-(4-(4-sulfamoylphenyl)-1H-1,2,3-triazol-1-yl)hexanoic acid
  SITE 2: note = 2-amino-3-((2S,3R,4S,5R,6S)-3,4,5,6-tetrahydroxytetrahydro-2H-pyran-2-carboxamido)propanoic acid
  SITE 4: note = 2-amino-3-((2S,3R,4S,5R,6S)-3,4,5,6-tetrahydroxytetrahydro-2H-pyran-2-carboxamido)propanoic acid
  SITE 7: note = (R)-2-amino-4-(4-(4-sulfamoylphenyl)-1H-1,2,3-triazol-1-yl)butanoic acid
  SITE 9: note = (R)-2-amino-4-(4-(4-sulfamoylphenyl)-1H-1,2,3-triazol-1-yl)butanoic acid; note = (R)-2-amino-4-(4-(4-sulfamoylphenyl)-1H-1,2,3-triazol-1-yl)butanoic acid is linked via an amide linkage to the carboxyl group of side chain in the Glutamic Acid at position 8.
  SITE 9: note = The (R)-2-amino-4-(4-(4-sulfamoylphenyl)-1H-1,2,3-triazol-1-yl)butanoic acid in position number 9 is linked via an amide linkage to another sequence.
XXSXRRXEX

SEQ ID NO: 99 - protein, 8 aa, synthetic construct
  REGION 1..8: note = Synthetic Polypeptide; note = (R)-2-amino-6-(4-(4-sulfamoylphenyl)-1H-1,2,3-triazol-1-yl)hexanoic acid at position 1 and Glutamic Acid at position 8 are linked via an amide linkage to form a cyclic peptide.
  SITE 1: note = (R)-2-amino-6-(4-(4-sulfamoylphenyl)-1H-1,2,3-triazol-1-yl)hexanoic acid
  SITE 2: note = (R)-2-amino-4-(4-(4-sulfamoylphenyl)-1H-1,2,3-triazol-1-yl)butanoic acid
  SITE 4: note = 2-amino-3-((2S,3R,4S,5R,6S)-3,4,5,6-tetrahydroxytetrahydro-2H-pyran-2-carboxamido)propanoic acid
  SITE 7: note = (R)-2-amino-4-(4-(4-sulfamoylphenyl)-1H-1,2,3-triazol-1-yl)butanoic acid
  SITE 8: note = The side chain of the glutamic acid in position number 8 is linked via an amide linkage to another sequence.
XXRXRSXE

SEQ ID NO: 100 - protein, 8 aa, synthetic construct
  REGION 1..8: note = Synthetic Polypeptide; note = (R)-2-amino-6-(4-(4-sulfamoylphenyl)-1H-1,2,3-triazol-1-yl)hexanoic acid at position 1 and Glutamic Acid at position 8 are linked via an amide linkage to form a cyclic peptide.
  SITE 1: note = (R)-2-amino-6-(4-(4-sulfamoylphenyl)-1H-1,2,3-triazol-1-yl)hexanoic acid
  SITE 2: note = (R)-2-amino-4-(4-(4-sulfamoylphenyl)-1H-1,2,3-triazol-1-yl)butanoic acid
  SITE 4: note = 2-amino-3-((2S,3R,4S,5R,6S)-3,4,5,6-tetrahydroxytetrahydro-2H-pyran-2-carboxamido)propanoic acid
  SITE 7: note = (R)-2-amino-4-(4-(4-sulfamoylphenyl)-1H-1,2,3-triazol-1-yl)butanoic acid
  SITE 8: note = The side chain of the glutamic acid in position number 8 is linked via an amide linkage to another sequence.
XXRXSRXE

SEQ ID NO: 101 - protein, 8 aa, synthetic construct
  REGION 1..8: note = (R)-2-amino-6-(4-(4-sulfamoylphenyl)-1H-1,2,3-triazol-1-yl)hexanoic acid at position 1 and Glutamic Acid at position 8 are linked via an amide linkage to form a cyclic peptide.; note = Synthetic Polypeptide
  SITE 1: note = (R)-2-amino-6-(4-(4-sulfamoylphenyl)-1H-1,2,3-triazol-1-yl)hexanoic acid
  SITE 2: note = (R)-2-amino-4-(4-(4-sulfamoylphenyl)-1H-1,2,3-triazol-1-yl)butanoic acid
  SITE 4: note = 2-amino-3-((2S,3R,4S,5R,6S)-3,4,5,6-tetrahydroxytetrahydro-2H-pyran-2-carboxamido)propanoic acid
  SITE 7: note = (R)-2-amino-4-(4-(4-sulfamoylphenyl)-1H-1,2,3-triazol-1-yl)butanoic acid
  SITE 8: note = The side chain of the glutamic acid in position number 8 is linked via an amide linkage to another sequence.
XXSXRRXE

SEQ ID NO: 102 - skipped

SEQ ID NO: 103 - protein, 8 aa, synthetic construct
  REGION 1..8: note = Synthetic Polypeptide; note = (R)-2-amino-6-(4-(4-sulfamoylphenyl)-1H-1,2,3-triazol-1-yl)hexanoic acid at position 1 and Glutamic Acid at position 8 are linked via an amide linkage to form a cyclic peptide.
  SITE 1: note = (R)-2-amino-6-(4-(4-sulfamoylphenyl)-1H-1,2,3-triazol-1-yl)hexanoic acid
  SITE 2: note = 2-amino-3-((2S,3R,4S,5R,6S)-3,4,5,6-tetrahydroxytetrahydro-2H-pyran-2-carboxamido)propanoic acid
  MOD_RES 4: note = N6-(2-(4-iodophenyl)acetyl)-D-lysine
  SITE 7: note = (R)-2-amino-6-(4-(4-sulfamoylphenyl)-1H-1,2,3-triazol-1-yl)hexanoic acid
  SITE 8: note = The side chain of the glutamic acid in position number 8 is linked via an amide linkage to another sequence.
XXRXRRXE

SEQ ID NO: 104 - protein, 8 aa, synthetic construct
  REGION 1..8: note = Synthetic Polypeptide; note = (R)-2-amino-6-(4-(4-sulfamoylphenyl)-1H-1,2,3-triazol-1-yl)hexanoic acid at position 1 and Glutamic Acid at position 8 are linked via an amide linkage to form a cyclic peptide.
  SITE 1: note = (R)-2-amino-6-(4-(4-sulfamoylphenyl)-1H-1,2,3-triazol-1-yl)hexanoic acid
  SITE 2: note = (R)-2-amino-4-(4-(4-sulfamoylphenyl)-1H-1,2,3-triazol-1-yl)butanoic acid
  MOD_RES 4: note = N6-(2-(4-iodophenyl)acetyl)-D-lysine
  SITE 7: note = (R)-2-amino-4-(4-(4-sulfamoylphenyl)-1H-1,2,3-triazol-1-yl)butanoic acid
  SITE 8: note = The side chain of the glutamic acid in position number 8 is linked via an amide linkage to another sequence.
XXRXRRXE

SEQ ID NO: 105 - protein, 9 aa, synthetic construct
  REGION 1..9: note = Synthetic Polypeptide
  REGION 1..8: note = (R)-2-amino-6-(4-(4-sulfamoylphenyl)-1H-1,2,3-triazol-1-yl)hexanoic acid at position 1 and Glutamic Acid at position 8 are linked via an amide linkage to form a cyclic peptide.
  SITE 1: note = (R)-2-amino-6-(4-(4-sulfamoylphenyl)-1H-1,2,3-triazol-1-yl)hexanoic acid
  SITE 4: note = 2-amino-3-((2S,3R,4S,5R,6S)-3,4,5,6-tetrahydroxytetrahydro-2H-pyran-2-carboxamido)propanoic acid
  SITE 7: note = (R)-2-amino-4-(4-(4-sulfamoylphenyl)-1H-1,2,3-triazol-1-yl)butanoic acid
  SITE 9: note = (R)-2-amino-4-(4-(4-sulfamoylphenyl)-1H-1,2,3-triazol-1-yl)butanoic acid; note = (R)-2-amino-4-(4-(4-sulfamoylphenyl)-1H-1,2,3-triazol-1-yl)butanoic acid is linked via an amide linkage to the carboxyl group of side chain in the Glutamic Acid at position 8.
  SITE 9: note = The (R)-2-amino-4-(4-(4-sulfamoylphenyl)-1H-1,2,3-triazol-1-yl)butanoic acid in position number 9 is linked via an amide linkage to another sequence.
XERXRRXEX

SEQ ID NO: 106 - protein, 8 aa, synthetic construct
  REGION 1..8: note = (R)-2-amino-6-(4-(4-sulfamoylphenyl)-1H-1,2,3-triazol-1-yl)hexanoic acid at position 1 and Glutamic Acid at position 8 are linked via an amide linkage to form a cyclic peptide.; note = Synthetic Polypeptide
  SITE 1: note = (R)-2-amino-6-(4-(4-sulfamoylphenyl)-1H-1,2,3-triazol-1-yl)hexanoic acid
  SITE 2: note = (R)-2-amino-4-(4-(4-sulfamoylphenyl)-1H-1,2,3-triazol-1-yl)butanoic acid
  SITE 7: note = (R)-2-amino-4-(4-(4-sulfamoylphenyl)-1H-1,2,3-triazol-1-yl)butanoic acid
  SITE 8: note = The side chain of the glutamic acid in position number 8 is linked via an amide linkage to another sequence.
XXSSSSXE

SEQ ID NO: 107 - protein, 8 aa, synthetic construct
  REGION 1..8: note = (R)-2-amino-6-(4-(4-sulfamoylphenyl)-1H-1,2,3-triazol-1-yl)hexanoic acid at position 1 and Glutamic Acid at position 8 are linked via an amide linkage to form a cyclic peptide.; note = Synthetic Polypeptide
  SITE 1: note = (R)-2-amino-6-(4-(4-sulfamoylphenyl)-1H-1,2,3-triazol-1-yl)hexanoic acid
  SITE 2: note = (R)-2-amino-4-(4-(4-sulfamoylphenyl)-1H-1,2,3-triazol-1-yl)butanoic acid
  SITE 4: note = 2-amino-3-((2S,3R,4S,5R,6S)-3,4,5,6-tetrahydroxytetrahydro-2H-pyran-2-carboxamido)propanoic acid
  SITE 7: note = (R)-2-amino-4-(4-(4-sulfamoylphenyl)-1H-1,2,3-triazol-1-yl)butanoic acid
  SITE 8: note = The side chain of the glutamic acid in position number 8 is linked via an amide linkage to another sequence.
XXSXRSXE